European Patent Specification EP 3 274 712 B1, published June 3, 2026. Title: LIPID-BINDING PROBES AND USES THEREOF. Applicant: THE SCRIPPS RESEARCH INSTITUTE. The sequence listing filed with the application follows.

SEQUENCE LISTING (122 sequences)

SEQ ID NO: 1 - protein, 21 aa, Mus musculus
ETPPDALILESPFTNIREEAK

SEQ ID NO: 2 - protein, 22 aa, Mus musculus
TIAILGAGHYVYADQPEEFNQK

SEQ ID NO: 3 - protein, 12 aa, Mus musculus
NNSIWDELFFNK

SEQ ID NO: 4 - protein, 16 aa, Mus musculus
ETTDTDTADQVIASFK

SEQ ID NO: 5 - protein, 36 aa, Mus musculus
FEAPEALFQPHLINVEGVGVAELLFNTIQAADIDTR

SEQ ID NO: 6 - protein, 21 aa, Mus musculus
HVDTAYAYQVEEEIGQAIQSK

SEQ ID NO: 7 - protein, 21 aa, Mus musculus
HVDTAYAYQVEEEIGQAIQSK

SEQ ID NO: 8 - protein, 28 aa, Mus musculus
VYLASLETLDNGKPFQESYVLDLDEVIK

SEQ ID NO: 9 - protein, 10 aa, Mus musculus
GYIVIEDLWK

SEQ ID NO: 10 - protein, 21 aa, Mus musculus
LGEIVTTIPTIGFNVETVEYK

SEQ ID NO: 11 - protein, 21 aa, Mus musculus
LGEIVTTIPTIGFNVETVEYK

SEQ ID NO: 12 - protein, 18 aa, Mus musculus
MLLEDELQDAVLLLFANK

SEQ ID NO: 13 - protein, 21 aa, Mus musculus
LGEIVTTIPTIGFNVETVEYK

SEQ ID NO: 14 - protein, 21 aa, Mus musculus
LGEIVTTIPTIGFNVETVEYK

SEQ ID NO: 15 - protein, 28 aa, Mus musculus
SSNLLAVETASLEEQLQGWGEVMLMADK

SEQ ID NO: 16 - protein, 8 aa, Mus musculus
AFVTDWDK

SEQ ID NO: 17 - protein, 26 aa, Mus musculus
NLEAVETLGSTSTICSDKTGTLTQNR

SEQ ID NO: 18 - protein, 26 aa, Mus musculus
NLEAVETLGSTSTICSDKTGTLTQNR

SEQ ID NO: 19 - protein, 19 aa, Mus musculus
VELVPPTPAEIPTAIQSVK

SEQ ID NO: 20 - protein, 14 aa, Mus musculus
YAEIVHLTLPDGTK

SEQ ID NO: 21 - protein, 7 aa, Mus musculus
YDDVTEK

SEQ ID NO: 22 - protein, 10 aa, Mus musculus
FLDELEDEAK

SEQ ID NO: 23 - protein, 15 aa, Mus musculus
SSLQTMESDVYTEVR

SEQ ID NO: 24 - protein, 21 aa, Mus musculus
TDFYDQCNDVGLMAYLGTITK

SEQ ID NO: 25 - protein, 14 aa, Mus musculus
NVFENPTMVQFDHR

SEQ ID NO: 26 - protein, 20 aa, Mus musculus
DGTAAVHFEHAWGDGVAVLR

SEQ ID NO: 27 - protein, 18 aa, Mus musculus
AIGAVPLIQGEYMIPCEK

SEQ ID NO: 28 - protein, 7 aa, Mus musculus
HFWADSK

SEQ ID NO: 29 - protein, 17 aa, Mus musculus
VFSSLGFSGTWECPELR

SEQ ID NO: 30 - protein, 14 aa, Mus musculus
NGDLPWPPLRNEFK

SEQ ID NO: 31 - protein, 16 aa, Mus musculus
DVLLTDFVPSMAVYIR

SEQ ID NO: 32 - protein, 26 aa, Mus musculus
YCTQDAFFQIKEVDMGLAADVGTLQR

SEQ ID NO: 33 - protein, 15 aa, Mus musculus
EVDMGLAADVGTLQR

SEQ ID NO: 34 - protein, 8 aa, Mus musculus
SLHMYLEK

SEQ ID NO: 35 - protein, 14 aa, Mus musculus
FYEQMNGPVTSGSR

SEQ ID NO: 36 - protein, 15 aa, Mus musculus
AMGPLVLTEVLFDEK

SEQ ID NO: 37 - protein, 29 aa, Mus musculus
SSLGLSYYPTSSTSSVSSSSSSPSSWLTR

SEQ ID NO: 38 - protein, 11 aa, Mus musculus
DCYPVQETFIR

SEQ ID NO: 39 - protein, 33 aa, Mus musculus
ESGYLHIQATKPDTVGCALNDSPVGLAAYILEK

SEQ ID NO: 40 - protein, 16 aa, Mus musculus
DIQQWEYVPLGPFLGK

SEQ ID NO: 41 - protein, 31 aa, Mus musculus
EVTVLGVATAPTQVLSNGIPVSNFTYSPDNK

SEQ ID NO: 42 - protein, 20 aa, Mus musculus
GLAFIQDPDGYWIEILNPNK

SEQ ID NO: 43 - protein, 23 aa, Mus musculus
VGDGAGGAFQPYLDSLRQELQQR

SEQ ID NO: 44 - protein, 14 aa, Mus musculus
MQLIMLCYNPDFEK

SEQ ID NO: 45 - protein, 14 aa, Mus musculus
IQLAMVCYSPDFEK

SEQ ID NO: 46 - protein, 13 aa, Mus musculus
YVTLIYTNYENGK

SEQ ID NO: 47 - protein, 22 aa, Mus musculus
LGAGYPMGPFELLDYVGLDTTK

SEQ ID NO: 48 - protein, 12 aa, Mus musculus
SSSDMPETITSR

SEQ ID NO: 49 - protein, 19 aa, Mus musculus
EGRPSGEAFVELESEDEVK

SEQ ID NO: 50 - protein, 19 aa, Mus musculus
EGRPSGEAFVELESEDEVK

SEQ ID NO: 51 - protein, 8 aa, Mus musculus
AQAYQTGK

SEQ ID NO: 52 - protein, 10 aa, Mus musculus
VYEGERPLTK

SEQ ID NO: 53 - protein, 21 aa, Mus musculus
LYGSGGPPPTGEEDTSEKDEL

SEQ ID NO: 54 - protein, 11 aa, Mus musculus
ELGENLDQILR

SEQ ID NO: 55 - protein, 16 aa, Mus musculus
NSNLVGAAHEELQQSR

SEQ ID NO: 56 - protein, 24 aa, Mus musculus
SLEGDLEDLKDQIAQLEASLSAAK

SEQ ID NO: 57 - protein, 23 aa, Mus musculus
SEAELATALSDKQGLETEVAELR

SEQ ID NO: 58 - protein, 13 aa, Mus musculus
GLWPGVEDLSLNK

SEQ ID NO: 59 - protein, 27 aa, Mus musculus
NTLVVSFADLEQFNQQLSTTIQEEFYR

SEQ ID NO: 60 - protein, 25 aa, Mus musculus
ASVPEGFLSELTQQLAQATGKPAQY

SEQ ID NO: 61 - protein, 12 aa, Mus musculus
AFKDDYVVSLVR

SEQ ID NO: 62 - protein, 21 aa, Mus musculus
VLQYYQESEKPEELGSVTVQK

SEQ ID NO: 63 - protein, 15 aa, Mus musculus
QGADTLAFMSLLEEK

SEQ ID NO: 64 - protein, 15 aa, Mus musculus
YLLETSGNLDGLEYK

SEQ ID NO: 65 - protein, 21 aa, Mus musculus
STEAPLIIRPDSGNPLDTVLK

SEQ ID NO: 66 - protein, 10 aa, Mus musculus
FYEEVHDLER

SEQ ID NO: 67 - protein, 21 aa, Mus musculus
QWQPDIEWAEQFSGAVMYPSK

SEQ ID NO: 68 - protein, 10 aa, Mus musculus
GAPYNALAGK

SEQ ID NO: 69 - protein, 16 aa, Mus musculus
TLAEIAKVELDNMPLR

SEQ ID NO: 70 - protein, 29 aa, Mus musculus
TFFILHDINSDGVLDEQELEALFTKELEK

SEQ ID NO: 71 - protein, 16 aa, Mus musculus
YLQEVINVLETDGHFR

SEQ ID NO: 72 - protein, 13 aa, Mus musculus
QVIEVLETDPHFR

SEQ ID NO: 73 - protein, 12 aa, Mus musculus
EFGEEALNSLQK

SEQ ID NO: 74 - protein, 18 aa, Mus musculus
VNDEHPAYLASDEITTVR

SEQ ID NO: 75 - protein, 18 aa, Mus musculus
LLLDEFLGYDDILMSSVK

SEQ ID NO: 76 - protein, 20 aa, Mus musculus
SAYNEGDYYHTVLWMEQVLK

SEQ ID NO: 77 - protein, 30 aa, Mus musculus
TGPAATTLSDTAAAESLVDSSEVTVIGFFK

SEQ ID NO: 78 - protein, 17 aa, Mus musculus
HNQLPLVIEFTEQTAPK

SEQ ID NO: 79 - protein, 17 aa, Mus musculus
EIVSFGSGYGGNSLLGK

SEQ ID NO: 80 - protein, 11 aa, Mus musculus
AVENYLIQMAR

SEQ ID NO: 81 - protein, 14 aa, Mus musculus
FYGPEGPYGVFAGR

SEQ ID NO: 82 - protein, 20 aa, Mus musculus
GDQPGASGDNDDDEPPPLPR

SEQ ID NO: 83 - protein, 14 aa, Mus musculus
FYGPAGPYGIFAGR

SEQ ID NO: 84 - protein, 18 aa, Mus musculus
LCSGPGAGEESPAATLPR

SEQ ID NO: 85 - protein, 7 aa, Mus musculus
VFESIGK

SEQ ID NO: 86 - protein, 13 aa, Mus musculus
NETGGGEGIEVLK

SEQ ID NO: 87 - protein, 22 aa, Mus musculus
ALIESGLGTDFSPDVGYNGYTR

SEQ ID NO: 88 - protein, 23 aa, Mus musculus
TQLMSMLMMNLESRPVIFEDVGR

SEQ ID NO: 89 - protein, 14 aa, Mus musculus
YKYGYEIPVDMLCK

SEQ ID NO: 90 - protein, 19 aa, Mus musculus
RFFPYYVYNIIGGLDEEGK

SEQ ID NO: 91 - protein, 10 aa, Mus musculus
LLANMVYQYK

SEQ ID NO: 92 - protein, 10 aa, Mus musculus
FGAVEAAMAK

SEQ ID NO: 93 - protein, 34 aa, Mus musculus
SHLGMFPQNSTSEANRDTETGTEASILGESGEYK

SEQ ID NO: 94 - protein, 16 aa, Mus musculus
AYLESEVAISEELVQK

SEQ ID NO: 95 - protein, 7 aa, Mus musculus
WLSQYID

SEQ ID NO: 96 - protein, 23 aa, Mus musculus
GVYIIGSSGFDSIPADLGVLYTR

SEQ ID NO: 97 - protein, 25 aa, Mus musculus
LLNLGLITESQAHTLEDEVAEALQK

SEQ ID NO: 98 - protein, 14 aa, Mus musculus
TVQIEASTVEIEER

SEQ ID NO: 99 - protein, 17 aa, Mus musculus
TTGMGAIYGMAQATIDR

SEQ ID NO: 100 - protein, 17 aa, Mus musculus
LKDFEPYLEILESYSTK

SEQ ID NO: 101 - protein, 17 aa, Mus musculus
YYGGAEVVDEIELLCQR

SEQ ID NO: 102 - protein, 21 aa, Mus musculus
IMGLDLPDGGHLTHGYMSDVK

SEQ ID NO: 103 - protein, 16 aa, Mus musculus
DVPASGMYFMTYEWLK

SEQ ID NO: 104 - protein, 31 aa, Mus musculus
AEQLEPLEYLVSAAEAGAMTLCITNPLWVTK

SEQ ID NO: 105 - protein, 8 aa, Mus musculus
YELPLVIK

SEQ ID NO: 106 - protein, 8 aa, Mus musculus
LILEQMQK

SEQ ID NO: 107 - protein, 30 aa, Mus musculus
DSNTVLLPSNPSDVTSMVAQAMGVYGALTK

SEQ ID NO: 108 - protein, 18 aa, Mus musculus
GQNDLMGTAEDFADQFLR

SEQ ID NO: 109 - protein, 13 aa, Mus musculus
LCLISTFLEDGIR

SEQ ID NO: 110 - protein, 16 aa, Mus musculus
SAFSNLFGGEPLSYTR

SEQ ID NO: 111 - protein, 23 aa, Mus musculus
IVDDCGGAFTMGTIGGGIFQAFK

SEQ ID NO: 112 - protein, 22 aa, Mus musculus
GKEDPWNSITSGALTGAILAAR

SEQ ID NO: 113 - protein, 13 aa, Mus musculus
TKEEDGREAVEFR

SEQ ID NO: 114 - protein, 20 aa, Mus musculus
LEQLNQYPDFNNYLIFVLTK

SEQ ID NO: 115 - protein, 20 aa, Mus musculus
FFLEEIQLGEELLAQGDYEK

SEQ ID NO: 116 - protein, 19 aa, Mus musculus
DLLEQMMAEMIGEFPDLHR

SEQ ID NO: 117 - protein, 9 aa, Mus musculus
YQFTPAFLR

SEQ ID NO: 118 - protein, 9 aa, Mus musculus
YQFTPAFLR

SEQ ID NO: 119 - protein, 25 aa, Mus musculus
NLDSLEEDLDFLRDQFTTTEVNMAR

SEQ ID NO: 120 - protein, 29 aa, Mus musculus
TAFDEAIAELDTLNEESYKDSTLIMQLLR

SEQ ID NO: 121 - protein, 29 aa, Mus musculus
AAFDDAIAELDTLSEESYKDSTLIMQLLR

SEQ ID NO: 122 - protein, 29 aa, Mus musculus
YDPSLKPPFDIGFEGIGEVVALGLSASAR